European Patent Specification EP 3 858 371 B1, published March 4, 2026. Title: Medicament for mitigating conditions and/or suppressing onset of peripheral neuropathy induced by anti-malignant tumor agent. Applicant: Asahi Kasei Pharma Corporation. The sequence listing filed with the application follows.

SEQUENCE LISTING (5 sequences)

SEQ ID NO: 1 - protein, 516 aa, human
MLGVLVLGALALAGLGFPAPAEPQPGGSQCVEHDCFALYPGPATFLNASQICDGLRGHLMTVRSSVAADVISLLLNGDGGVGRRRLWIGLQLPPGCGDPKRLGPLRGFQWVTGDNNTSYSRWARLDLNGAPLCGPLCVAVSAAEATVPSEPIWEEQQCEVKADGFLCEFHFPATCRPLAVEPGAAAAAVSITYGTPFAARGADFQALPVGSSAAVAPLGLQLMCTAPPGAVQGHWAREAPGAWDCSVENGGCEHACNAIPGAPRCQCPAGAALQADGRSCTASATQSCNDLCEHFCVPNPDQPGSYSCMCETGYRLAADQHRCEDVDDCILEPSPCPQRCVNTQGGFECHCYPNYDLVDGECVEPVDPCFRANCEYQCQPLNQTSYLCVCAEGFAPIPHEPHRCQMFCNQTACPADCDPNTQASCECPEGYILDDGFICTDIDECENGGFCSGVCHNLPGTFECICGPDSALVRHIGTDCDSGKVDGGDSGSGEPPPSPTPGSTLTPPAVGLVHSG

SEQ ID NO: 2 - DNA, 1548 bp, human
atgcttggggtcctggtccttggcgcgctggccctggccggcctggggttccccgcacccgcagagccgcagccgggtggcagccagtgcgtcgagcacgactgcttcgcgctctacccgggccccgcgaccttcctcaatgccagtcagatctgcgacggactgcggggccacctaatgacagtgcgctcctcggtggctgccgatgtcatttccttgctactgaacggcgacggcggcgttggccgccggcgcctctggatcggcctgcagctgccacccggctgcggcgaccccaagcgcctcgggcccctgcgcggcttccagtgggttacgggagacaacaacaccagctatagcaggtgggcacggctcgacctcaatggggctcccctctgcggcccgttgtgcgtcgctgtctccgctgctgaggccactgtgcccagcgagccgatctgggaggagcagcagtgcgaagtgaaggccgatggcttcctctgcgagttccacttcccagccacctgcaggccactggctgtggagcccggcgccgcggctgccgccgtctcgatcacctacggcaccccgttcgcggcccgcggagcggacttccaggcgctgccggtgggcagctccgccgcggtggctcccctcggcttacagctaatgtgcaccgcgccgcccggagcggtccaggggcactgggccagggaggcgccgggcgcttgggactgcagcgtggagaacggcggctgcgagcacgcgtgcaatgcgatccctggggctccccgctgccagtgcccagccggcgccgccctgcaggcagacgggcgctcctgcaccgcatccgcgacgcagtcctgcaacgacctctgcgagcacttctgcgttcccaaccccgaccagccgggctcctactcgtgcatgtgcgagaccggctaccggctggcggccgaccaacaccggtgcgaggacgtggatgactgcatactggagcccagtccgtgtccgcagcgctgtgtcaacacacagggtggcttcgagtgccactgctaccctaactacgacctggtggacggcgagtgtgtggagcccgtggacccgtgcttcagagccaactgcgagtaccagtgccagcccctgaaccaaactagctacctctgcgtctgcgccgagggcttcgcgcccattccccacgagccgcacaggtgccagatgttttgcaaccagactgcctgtccagccgactgcgaccccaacacccaggctagctgtgagtgccctgaaggctacatcctggacgacggtttcatctgcacggacatcgacgagtgcgaaaacggcggcttctgctccggggtgtgccacaacctccccggtaccttcgagtgcatctgcgggcccgactcggcccttgtccgccacattggcaccgactgtgactccggcaaggtggacggtggcgacagcggctctggcgagcccccgcccagcccgacgcccggctccaccttgactcctccggccgtggggctcgtgcattcgggc

SEQ ID NO: 3 - protein, 516 aa, human
MLGVLVLGALALAGLGFPAPAEPQPGGSQCVEHDCFALYPGPATFLNASQICDGLRGHLMTVRSSVAADVISLLLNGDGGVGRRRLWIGLQLPPGCGDPKRLGPLRGFQWVTGDNNTSYSRWARLDLNGAPLCGPLCVAVSAAEATVPSEPIWEEQQCEVKADGFLCEFHFPATCRPLAVEPGAAAAAVSITYGTPFAARGADFQALPVGSSAAVAPLGLQLMCTAPPGAVQGHWAREAPGAWDCSVENGGCEHACNAIPGAPRCQCPAGAALQADGRSCTASATQSCNDLCEHFCVPNPDQPGSYSCMCETGYRLAADQHRCEDVDDCILEPSPCPQRCVNTQGGFECHCYPNYDLVDGECVEPVDPCFRANCEYQCQPLNQTSYLCVCAEGFAPIPHEPHRCQMFCNQTACPADCDPNTQASCECPEGYILDDGFICTDIDECENGGFCSGVCHNLPGTFECICGPDSALARHIGTDCDSGKVDGGDSGSGEPPPSPTPGSTLTPPAVGLVHSG

SEQ ID NO: 4 - DNA, 1548 bp, human
atgcttggggtcctggtccttggcgcgctggccctggccggcctggggttccccgcacccgcagagccgcagccgggtggcagccagtgcgtcgagcacgactgcttcgcgctctacccgggccccgcgaccttcctcaatgccagtcagatctgcgacggactgcggggccacctaatgacagtgcgctcctcggtggctgccgatgtcatttccttgctactgaacggcgacggcggcgttggccgccggcgcctctggatcggcctgcagctgccacccggctgcggcgaccccaagcgcctcgggcccctgcgcggcttccagtgggttacgggagacaacaacaccagctatagcaggtgggcacggctcgacctcaatggggctcccctctgcggcccgttgtgcgtcgctgtctccgctgctgaggccactgtgcccagcgagccgatctgggaggagcagcagtgcgaagtgaaggccgatggcttcctctgcgagttccacttcccagccacctgcaggccactggctgtggagcccggcgccgcggctgccgccgtctcgatcacctacggcaccccgttcgcggcccgcggagcggacttccaggcgctgccggtgggcagctccgccgcggtggctcccctcggcttacagctaatgtgcaccgcgccgcccggagcggtccaggggcactgggccagggaggcgccgggcgcttgggactgcagcgtggagaacggcggctgcgagcacgcgtgcaatgcgatccctggggctccccgctgccagtgcccagccggcgccgccctgcaggcagacgggcgctcctgcaccgcatccgcgacgcagtcctgcaacgacctctgcgagcacttctgcgttcccaaccccgaccagccgggctcctactcgtgcatgtgcgagaccggctaccggctggcggccgaccaacaccggtgcgaggacgtggatgactgcatactggagcccagtccgtgtccgcagcgctgtgtcaacacacagggtggcttcgagtgccactgctaccctaactacgacctggtggacggcgagtgtgtggagcccgtggacccgtgcttcagagccaactgcgagtaccagtgccagcccctgaaccaaactagctacctctgcgtctgcgccgagggcttcgcgcccattccccacgagccgcacaggtgccagatgttttgcaaccagactgcctgtccagccgactgcgaccccaacacccaggctagctgtgagtgccctgaaggctacatcctggacgacggtttcatctgcacggacatcgacgagtgcgaaaacggcggcttctgctccggggtgtgccacaacctccccggtaccttcgagtgcatctgcgggcccgactcggcccttgcccgccacattggcaccgactgtgactccggcaaggtggacggtggcgacagcggctctggcgagcccccgcccagcccgacgcccggctccaccttgactcctccggccgtggggctcgtgcattcgggc

SEQ ID NO: 5 - DNA, 21 bp, Artificial Sequence
  Description of Artificial Sequence: Synthetic DNA
aatgtggcgggcaagggccga